European Patent Application EP 4 382 134 A1, published June 12, 2024. Title: PHARMACEUTICAL COMPOSITION FOR PREVENTING OR TREATING TRIPLE-NEGATIVE BREAST CANCER, COMPRISING OLIGONUCLEOTIDE AS ACTIVE INGREDIENT. Applicant: Interoligo Corporation. Application EP 22853571.2, filed August 5, 2022. The sequence listing filed with the application follows.

SEQUENCE LISTING (30 sequences)

SEQ ID NO: 1 - skipped

SEQ ID NO: 2 - DNA, 12 bp, synthetic construct
  source 1..12: mol_type = other DNA
tggttgtggtgg

SEQ ID NO: 3 - DNA, 12 bp, synthetic construct
  source 1..12: mol_type = other DNA
tggtggttgtgg

SEQ ID NO: 4 - DNA, 15 bp, synthetic construct
  source 1..15: mol_type = other DNA
tggtggttgtggtgg

SEQ ID NO: 5 - DNA, 18 bp, synthetic construct
  source 1..18: mol_type = other DNA
tggtggttgtggtggtgg

SEQ ID NO: 6 - DNA, 18 bp, synthetic construct
  source 1..18: mol_type = other DNA
tggtggtggttgtggtgg

SEQ ID NO: 7 - DNA, 21 bp, synthetic construct
  source 1..21: mol_type = other DNA
tggtggtggttgtggtggtgg

SEQ ID NO: 8 - DNA, 24 bp, synthetic construct
  source 1..24: mol_type = other DNA
tggtggtggttgtggtggtggtgg

SEQ ID NO: 9 - DNA, 24 bp, synthetic construct
  source 1..24: mol_type = other DNA
tggtggtggtggttgtggtggtgg

SEQ ID NO: 10 - DNA, 27 bp, synthetic construct
  source 1..27: mol_type = other DNA
tggtggtggtggttgtggtggtggtgg

SEQ ID NO: 11 - DNA, 30 bp, synthetic construct
  source 1..30: mol_type = other DNA
tggtggtggtggttgtggtggtggtggtgg

SEQ ID NO: 12 - DNA, 30 bp, synthetic construct
  source 1..30: mol_type = other DNA
tggtggtggtggtggttgtggtggtggtgg

SEQ ID NO: 13 - DNA, 33 bp, synthetic construct
  source 1..33: mol_type = other DNA
tggtggtggtggtggttgtggtggtggtggtgg

SEQ ID NO: 14 - DNA, 36 bp, synthetic construct
  source 1..36: mol_type = other DNA
tggtggtggtggtggttgtggtggtggtggtggtgg

SEQ ID NO: 15 - DNA, 36 bp, synthetic construct
  source 1..36: mol_type = other DNA
tggtggtggtggtggtggttgtggtggtggtggtgg

SEQ ID NO: 16 - DNA, 39 bp, synthetic construct
  source 1..39: mol_type = other DNA
tggtggtggtggtggtggttgtggtggtggtggtggtgg

SEQ ID NO: 17 - DNA, 42 bp, synthetic construct
  source 1..42: mol_type = other DNA
tggtggtggtggtggtggttgtggtggtggtggtggtggtgg

SEQ ID NO: 18 - DNA, 42 bp, synthetic construct
  source 1..42: mol_type = other DNA
tggtggtggtggtggtggtggttgtggtggtggtggtggtgg

SEQ ID NO: 19 - DNA, 45 bp, synthetic construct
  source 1..45: mol_type = other DNA
tggtggtggtggtggtggtggttgtggtggtggtggtggtggtgg

SEQ ID NO: 20 - DNA, 48 bp, synthetic construct
  source 1..48: mol_type = other DNA
tggtggtggtggtggtggtggttgtggtggtggtggtggtggtggtgg

SEQ ID NO: 21 - DNA, 48 bp, synthetic construct
  source 1..48: mol_type = other DNA
tggtggtggtggtggtggtggtggttgtggtggtggtggtggtggtgg

SEQ ID NO: 22 - DNA, 51 bp, synthetic construct
  source 1..51: mol_type = other DNA
tggtggtggtggtggtggtggtggttgtggtggtggtggtggtggtggtgg

SEQ ID NO: 23 - DNA, 54 bp, synthetic construct
  source 1..54: mol_type = other DNA
tggtggtggtggtggtggtggtggttgtggtggtggtggtggtggtggtggtgg

SEQ ID NO: 24 - DNA, 54 bp, synthetic construct
  source 1..54: mol_type = other DNA
tggtggtggtggtggtggtggtggtggttgtggtggtggtggtggtggtggtgg

SEQ ID NO: 25 - DNA, 57 bp, synthetic construct
  source 1..57: mol_type = other DNA
tggtggtggtggtggtggtggtggtggttgtggtggtggtggtggtggtggtggtgg

SEQ ID NO: 26 - DNA, 60 bp, synthetic construct
  source 1..60: mol_type = other DNA
tggtggtggtggtggtggtggtggtggttgtggtggtggtggtggtggtggtggtggtgg

SEQ ID NO: 27 - DNA, 60 bp, synthetic construct
  source 1..60: mol_type = other DNA
tggtggtggtggtggtggtggtggtggtggttgtggtggtggtggtggtggtggtggtgg

SEQ ID NO: 28 - DNA, 63 bp, synthetic construct
  source 1..63: mol_type = other DNA
tggtggtggtggtggtggtggtggtggtggttgtggtggtggtggtggtggtggtggtggtgg

SEQ ID NO: 29 - DNA, 32 bp, synthetic construct
  source 1..32: mol_type = other DNA
  modified_base 1: mod_base = OTHER; note = 2', 2'-difluoro deoxycytidine
  modified_base 2: mod_base = OTHER; note = 2', 2'-difluoro deoxycytidine
nntggtggtggtggttgtggtggtggtggtgg

SEQ ID NO: 30 - DNA, 29 bp, synthetic construct
  source 1..29: mol_type = other DNA
  modified_base 1: mod_base = OTHER; note = 2', 2'-difluoro deoxycytidine
  modified_base 2: mod_base = OTHER; note = 2', 2'-difluoro deoxycytidine
nntcctcctcctccttctcctcctcctcc